European Patent Application EP 4 112 053 A1, published January 4, 2023. Title: Treatment of synucleinopathies. Applicant: Deutsches Zentrum für Neurodegenerative Erkrankungen (DZNE) Klinikum rechts der Isar der Technischen Universität München. The sequence listing filed with the application follows.

SEQUENCE LISTING (4 sequences)

SEQ ID NO: 1 - RNA, 25 nt, Artificial Sequence
  siRNA Sequences against PDE1A sense
ccagcagcugucaucguaacauuaa

SEQ ID NO: 2 - RNA, 25 nt, Artificial Sequence
  siRNA Sequences against PDE1A antisense
uuaauguuacgaugacagcugcugg

SEQ ID NO: 3 - RNA, 25 nt, Artificial Sequence
  siRNA Sequences against PDE1C sense
caccagcuguuauugaggcauuaaa

SEQ ID NO: 4 - RNA, 25 nt, Artificial Sequence
  siRNA Sequences against PDE1C antisense
uuuaaugccucaauaacagcuggug